European Patent Specification EP 3 323 820 B1, published May 10, 2023. Title: SUBSTITUTED 6,5-FUSED BICYCLIC HETEROARYL COMPOUNDS. Applicant: EPIZYME, INC. KUNTZ, Kevin  W OLHAVA, Edward  J CHESWORTH, Richard DUNCAN, Kenneth  W. The sequence listing filed with the application follows.

SEQUENCE LISTING (2 sequences)

SEQ ID NO: 1 - protein, 26 aa, Artificial Sequence
  Chemically synthesized polypeptide
  MISC_FEATURE (26)..(26): wherein a biotin and an amide are conjugated
ATKAARKSAPATGGVKKPHRYRPGGK

SEQ ID NO: 2 - protein, 26 aa, Artificial Sequence
  Chemically synthesized polypeptide
  MISC_FEATURE (7)..(7): wherein the lysine is dimethylated
  MISC_FEATURE (26)..(26): wherein a biotin and an amide are conjugated
ATKAARKSAPATGGVKKPHRYRPGGK